European Patent Application EP 4 501 345 A1, published February 5, 2025. Title: A Composition Comprising Aflibercept and a Variant thereof, and Related Methods and Uses. Applicant: QILU PHARMACEUTICAL CO., LTD. The sequence listing filed with the application follows.

SEQUENCE LISTING (4 sequences)

SEQ ID NO: 1 - protein, 432 aa, synthetic construct
SDTGRPFVEMYSEIPEIIHMTEGRELVIPCRVTSPNITVTLKKFPLDTLIPDGKRIIWDSRKGFIISNATYKEIGLLTCEATVNGHLYKTNYLTHRQTNTIIDVVLSPSHGIELSVGEKLVLNCTARTELNVGIDFNWEYPSSKHQHKKLVNRDLKTQSGSEMKKFLSTLTIDGVTRSDQGLYTCAASSGLMTKKNSTFVRVHEKDKTHTCPPCPAPELLGGPSVFLFPPKPKDTLMISRTPEVTCVVVDVSHEDPEVKFNWYVDGVEVHNAKTKPREEQYNSTYRVVSVLTVLHQDWLNGKEYKCKVSNKALPAPIEKTISKAKGQPREPQVYTLPPSRDELTKNQVSLTCLVKGFYPSDIAVEWESNGQPENNYKTTPPVLDSDGSFFLYSKLTVDKSRWQQGNVFSCSVMHEALHNHYTQKSLSLSPGK

SEQ ID NO: 2 - protein, 333 aa, synthetic construct
TIIDVVLSPSHGIELSVGEKLVLNCTARTELNVGIDFNWEYPSSKHQHKKLVNRDLKTQSGSEMKKFLSTLTIDGVTRSDQGLYTCAASSGLMTKKNSTFVRVHEKDKTHTCPPCPAPELLGGPSVFLFPPKPKDTLMISRTPEVTCVVVDVSHEDPEVKFNWYVDGVEVHNAKTKPREEQYNSTYRVVSVLTVLHQDWLNGKEYKCKVSNKALPAPIEKTISKAKGQPREPQVYTLPPSRDELTKNQVSLTCLVKGFYPSDIAVEWESNGQPENNYKTTPPVLDSDGSFFLYSKLTVDKSRWQQGNVFSCSVMHEALHNHYTQKSLSLSPGK

SEQ ID NO: 3 - protein, 432 aa, synthetic construct
SDTGRPFVEMYSEIPEIIHMTEGRELVIPCRVTSPNITVTLKKFPLDTLIPDGKRIIWDSRKGFIISNATYKEIGLLTCEATVNGHLYKTNYLTHRQTNTIIDVVLSPSHGIELSVGEKLVLNCTARTELNVGIDFNWEYPSSKHQHKKLVNRDLKTQSGSEMKKFLSTLTIDGVTRSDQGLYTCAASSGLMTKKNSTFVRVHEKDKTHTCPPCPAPELLGGPSVFLFPPKPKDTLMISRTPEVTCVVVDVSHEDPEVKFNWYVDGVEVHNAKTKPREEQYNSTYRVVSVLTVLHQDWLNGKEYKCKVSNKALPAPIEKTISKAKGQPREPQVYTLPPCRDELTKNQVSLWCLVKGFYPSDIAVEWESNGQPENNYKTTPPVLDSDGSFFLYSKLTVDKSRWQQGNVFSCSVMHEALHNHYTQKSLSLSPGK

SEQ ID NO: 4 - protein, 333 aa, synthetic construct
TIIDVVLSPSHGIELSVGEKLVLNCTARTELNVGIDFNWEYPSSKHQHKKLVNRDLKTQSGSEMKKFLSTLTIDGVTRSDQGLYTCAASSGLMTKKNSTFVRVHEKDKTHTCPPCPAPELLGGPSVFLFPPKPKDTLMISRTPEVTCVVVDVSHEDPEVKFNWYVDGVEVHNAKTKPREEQYNSTYRVVSVLTVLHQDWLNGKEYKCKVSNKALPAPIEKTISKAKGQPREPQVCTLPPSRDELTKNQVSLSCAVKGFYPSDIAVEWESNGQPENNYKTTPPVLDSDGSFFLVSKLTVDKSRWQQGNVFSCSVMHEALHNRYTQKSLSLSPGK